European Patent Specification EP 3 230 456 B1, published May 22, 2024. Title: Compositions and Methods for Controlling Plant Pests. Applicant: Syngenta Participations AG Bramlett, Matthew Richard Seguin, Katherine Kramer, Vance Cary Rose, Mark Scott. The sequence listing filed with the application follows.

SEQUENCE LISTING (26 sequences)

SEQ ID NO: 1 - DNA, 3444 bp, Bacillus thuringiensis
atggatttagacggtaataaaactgaaactgagactgaaattgtaaatggttccgaaagtagtatcgatccatcaagcgtgtcttatgcgggaaataacagctattcttccgctttgaatctcaattcttgtcaaaacagagggattgcacagtgggttaatacgcttggaggtgcaatcggtcaggctgtatccataggaacatccatcatttccttgcttgcggcgcctacgcttactggaagtatttcgttagcttttaatcttataaggagaatggggacaggcagtaatggaagctctatttcggacttgtcaatatgtgacttactatccataattaatttacgtgtaagtcaagctgtattgaacgacgggattgcagattttaacggctcagtggctgtatatgatctctatttgcatgctttacgcagttggaacaataaccctaatgctgctaccgcggaggaacttcgcactcgttttcgtattgcagattccgaattcgaacgtatcttaacgcgggggtccttgacacatggtggttcattagctagacaagatgctcaagtgttactgttaccttcttttgtaaatgctgcctatcttcatttacttatattaagggatgctagcagatatggggctagctggggcttgtttaatacgacaccacatatcaattatccagtaagattacaacaacttattggttcttatacccattactgcacacattggtataatcaaggtttaaatgaaatcagacaacgaggcaatacggctgtcaattggttggaatttcatagatacagaagagatatgacattaatggtactagatgttgtgtcattattttcagcgcttgatactataaggtatccgaacgcaaccgttgtccaattaagcagaaccgtttatacagacccgattggttttgtaaatcgtggaagcggcaacagattaagctggtttgattggcggaatcaagctaatttttcaacgctagaaagtgaaatgccaaccccctcgtctccactttctttgaatcatatgagtatatttacgggtccccttactttacctgtctctcctaatacccatagagccagggtatggtatggcaatcaaaatatgttcacaacgggtagtcaaaattcaggtcaaacaacaaactctattcaaaacatttcgggtttagaaatatttagaatagattctcaagcctgtaatctaaacaataattcgtatggcgtgaaccgagctgaattttttcatggcgctagtcagggctcccaaagatctgtttatcaaggctatattagacaaagtggattggacaacccggtagttatgaatcttcaaagctttttacctggcgaaaattcagcgacaccaaccgcacaagattatacgcatatattaagtaatcctgttaatataagaggaggacttcgacaaatagtagctgatcgtcgttcttctgtagtcgtttatggttggacacacaaaagtttgagtcgacgtagtttagttgcaccagatcaaattactcaagtacctgctgttaaagcaagtccctcatcccattgtaccatcattgcaggacctggatttacgggcggggatctcgtaagtctgcaaccaaatggacaactcgttataccgtttcaggtatcggcgccagaaacaaattatcatattcgaatatgttatgtttctacgtccgactgttccataaatacaatatgtaatgatgagacccatttaagtacgttgccttccacaacctcatcacttgaaaatttacaatgtaaccatttgcattattttaacgtgggcactttcaaacctacgatagatagtaaactaacgcttgtaaatacaagtccaaatgcaaatattatcatcgacaaaattgaatttattcccgtagatacggcccaacaacaaaatgaggatctagaagcagcaaaaaaagcggtggcgagcttgtttacacgcacaagggacggattacaagtaaatgtgaaagattatcaagtcgatcaagcggcaaatttagtgtcatgcttatcagatgaacaatatgggtatgacaaaaagatgttattggaagcggtacgtgcggcaaaacgacttagccgagaacgcaacttacttcaggacccagattttaatacaatcaatagtacagaagaaaatggatggaaagcaagtaacggcgttactattagtgagggcgggccattctataaaggccgtgcaattcagctagcaagtgcacgagaaaattacccaacatacatctatcaaaaagtagatgcatcggagttaaagccgtatacacgttatagactggatgggttcgtgaagagtagtcaagatttagaaattgatctcattcaccatcataaagtccatcttgtgaaaaatgtaccagataatttagtatctgatacttacccagatgattcttgtagtggaatcaatcgatgtcaggaacaacagatggtaaatgcgcaactggaaacagagcatcatcatccgatggattgctgtgaagcagctcaaacacatgagttttcttcctatattgatacaggggatttaaattcgagtgtagaccagggaatctgggcgatctttaaagttcgaacaaccgatggttatgcgacgttaggaaatcttgaattggtagaggtcggaccgttatcgggtgaatctttagaacgtgaacaaagggataatacaaaatggagtgcagagctaggaagaaagcgtgcagaaacagatcgcgtgtatcaagatgccaaacaatccatcaatcatttatttgtggattatcaagatcaacaattaaatccagaaatagggatggcagatattatggacgctcaaaatcttgtcgcatcaatttcagatgtatatagcgatgccgtactgcaaatccctggaattaactatgagatttacacagagctgtccaatcgcttacaacaagcatcgtatctgtatacgtctcgaaatgcggtgcaaaatggggactttaacaacgggctagatagctggaatgcaacagcgggtgcatcggtacaacaggatggcaatacgcatttcttagttctttctcattgggatgcacaagtttctcaacaatttagagtgcagccgaattgtaaatatgtattacgtgtaacagcagagaaagtaggcggcggagacggatacgtgactatccgggatgatgctcatcatacagaaacgcttacatttaatgcatgtgattatgatataaatggcacgtacgtgactgataatacgtatctaacaaaagaagtggtattccatccggagacacaacacatgtgggtagaggtaaatgaaacagaaggtgcatttcatatagatagtattgaattcgttgaaacagaaaagtaa

SEQ ID NO: 2 - DNA, 3474 bp, Bacillus thuringiensis
atgaatcgaaataatcaaaatgaatatgaaattattgatgccccccattgtgggtgtccatcagatgacgatgtgaagtatcctttggcaagtgacccaaatgcagcgttacaaaatatgaactataaagattacttacaaatgacagatgaggactacactgattcttatataaatcctagtttatctattagtggtagagatgcagttcagactgcgcttactgttgttgggagaatactcggggctttaggtgttccgttttctggacaaatagtgagtttttatcaattccttttaaatacactgtggccagttaatgatacagctatatgggaagctttcatgcgacaggtggaggaacttgtcaatcaacaaataacagaatttgcaagaaatcaggcacttgcaagattgcaaggattaggagattcttttaatgtatatcaacgttcccttcaaaattggttggctgatcgaaatgatacacgaaatttaagtgttgttcgtgctcaatttatagctttagaccttgattttgttaatgctattccattgtttgcagtaaatggacagcaggttccattactgtcagtatatgcacaagctgtgaatttacatttgttattattaaaagatgcatctctttttggagaaggatggggattcacacagggggaaatttccacatattatgaccgtcaattggaactaaccgctaggtacactaattactgtgaaacttggtataatacaggtttagatcgtttaagaggaacaaatactgaaagttggttaagatatcatcaattccgtagagaaatgactttagtggtattagatgttgtggcgctatttccatattatgatgtacgactttatccaacgggatcaaacccacagcttacacgtgaggtatatacagatccgattgtatttaatccaccagctaatgttggactttgccgacgttggggtactaatccctataatactttttctgagctcgaaaatgccttcattcgcccaccacatctttttgataggctgaatagcttaacaatcagcagtaatcgatttccagtttcatctaattttatggattattggtcaggacatacgttacgccgtagttatctgaacgattcagcagtacaagaagatagttatggcctaattacaaccacaagagcaacaattaatcccggagttgatggaacaaaccgcatagagtcaacggcagtagattttcgttctgcattgataggtatatatggcgtgaatagagcttcttttgtcccaggaggcttgtttaatggtacgacttctcctgctaatggaggatgtagagatctctatgatacaaatgatgaattaccaccagatgaaagtaccggaagttcaacccatagactatctcatgttaccttttttagctttcaaactaatcaggctggatctatagctaatgcaggaagtgtacctacttatgtttggacccgtcgtgatgtggaccttaataatacgattaccccaaatagaattacacaattaccattggtaaaggcatctgcacctgtttcgggtactacggtcttaaaaggtccaggatttacaggagggggtatactccgaagaacaactaatggcacatttggaacgttaagagtaacggttaattcaccattaacacaacaatatcgcctaagagttcgttttgcctcaacaggaaatttcagtataaggttactccgtggaggggtttctatcggtgatgttagattagggagcacaatgaacagagggcaggaactaacttacgaatcctttttcacaagagagtttactactactggtccgttcaatccgccttttacatttacacaagctcaagagattctaacagtgaatgcagaaggtgttagcaccggtggtgaatattatatagatagaattgaaattgtccctgtgaatccggcacgagaagcggaagaggatttagaagcggcgaagaaagcggtggcgagcttgtttacacgtacaagagatggattacaggtaaatgtgacagattaccaagtggatcgagcggcaaatttagtgtcatgcttatcagatgaacaatattcgcatgataaaaagatgttattggaagccgtacgcgcagcaaaacgcctcagccgcgaacgcaacttacttcaagatccagattttaatacaatcaatagtacagaagaaaatggctggaaggcaagtaacggtgttactattagcgagggcggtccattctttaaaggtcgtgcacttcagttagcaagcgcaagagaaaattatccaacatacatttatcaaaaagtagatgcatcggtgttaaagccttatacacgctatagactagatggatttgtgaagagtagtcaagatttagaaattgatctcatccaccatcataaagtccatcttgtaaaaaatgtaccagataatttagtatctgatacttactcagatggttcttgcagcggaatcaaccgttgtgatgaacagcagcaggtagatatgcagctagatgcggagcatcatccaatggattgctgtgaagcggctcaaacacatgagttttcttcctatattaatacaggggatctaaatgcaagtgtagatcagggcatttgggttgtattaaaagttcgaacaacagatgggtatgcgacgttaggaaatcttgaattggtagaggttgggccattatcgggtgaatctctagaacgcgaacaaagagataatgcgaaatggaatgcagagctaggaagaaagcgtgcagaaacagatcgcgtgtatctagctgcgaaacaagcaattaatcatctatttgtagactatcaagatcaacaattaaatccagaaattgggctagcggaaataaatgaagcttcaaatcttgtgaagtcaatttcgggtgtatatagtgatacactattacagattcctggaattaactacgaaatttacacagagttatccgatcgattacaacaagcatcgtatctgtatacgtctcgaaatgccgtgcaaaatggagactttaacagtggtctagatagttggaatgcaacaacagatgcatcggttcagcaagatggcagtacacatttcttagttctttcgcattgggatgcacaagtttcccaacaaatgagagtaaatttgaattgtaagtatgttttacgtgtaacagcaaaaaaagtaggaggcggagatggatacgtcacaatccgagatggcgctcatcaccaagaaactcttacatttaatgcatgtgactacgatgtaaatggtacgtatgtcaatgacaattcgtacataacaaaagaagtggtattctacccagagacaaaacatatgtgggtagaggtgagtgaatccgaaggttcattctatatagacagtattgagtttattgaaacacaagagtag

SEQ ID NO: 3 - DNA, 3522 bp, Bacillus thuringiensis
atgaatcgaaataatcaaggtgaatatgaaattattgacgcttccacttgtggttgttcgtcagatgatgttgttcaatatcctttggcaagagatccgaatgctgcattccaaaatatgaattataaagattatttgaaaatgtctgacggagactacgtcgattcttatataaacccaggcttatctattggtcgtagagatgtgaccctaactggagttggtattgttgcgctaatagtagggactttaggtggtccagttgggggtatagtaactggcttgatttcctctcttttaggattattgtggccaagtaatgataatgatgtatgggaagcttttatggcacaaatagaagagctaattgaacaaaggatagcagatcaagtagtaaggaatgcactcgataacttaactggattgcgcgattattataatcaatacctattagcattggaggagtggcaggaaaggccgaacgctgtaagatctaccttagtttttaatagatttgaaaccctgcattctcactttgtaactagtatgccaagctttggtagtggccctggaagtgaaaggtatgcggtacaattgctgacagtttatgcacaagcggcaaatctgcatttgttattattaagagatgctgacatttatggggcaaggtggggacttcgtgaatctcagattgatttatattttaatgagctacaaaatcgtactcgagattataccaatcattgtgtaactgcgtacaataatgggttagaggagatacgaggaacaagccctgcaagttggttgaggtaccatcaattccgtagagagacaacactaatagcattggatttagtggcgatattcccatattacaacgtacgagaatatccaattggggtaaatcctcagcttacacgtgatgtatatacagatccaataggggttactttcagaagagaagattgggaaacaggagtagaatgcagaccatgggtaaatactccttacatgagcttttcggatcttgaaaatgcaataattcgtccaccacatctatttgaaacattacgtaatttaacaattcatacaggtcgatataacctagtaggaggggcgagatttattgaaggatgggtcggacattctgtaacaaatactcgcttgggtaattcaacagtatttacaagtaattatggttctttgccacctcgttttcaagtttttaattttactaattttgatgtttaccaaattaatacgagagcagattctacaggtacctttagaatccctggatttgcagttacaagggcccaattcattccgggtgggacttattcagtagctcaccgagatccaggggcatgtcaacaagattatgattcaattgaagagttaccaagtctagacccggatgaacctattaatagaagttatagtcatagattatcgcatgttaccctttataaatatactctctcagatacagattatggagttatcaattatacagattatggaagtatgcctgcatatgtctggacacatcgcgatgtggaccttactaacacgattactgcagatagaattacacaactcccattagtaaaggcatctacactacctgcgggtactactgtggtaaaaggcccaggatttacaggaggagatatactccgaagaacaactaatggaacatttgggacattacatgtaagggttaattcaccattaacacaacaatatcgcctaagagttcgttttgcctcaacaggaaatttcagtataagggtactccgtggagggacttctatcggtgatgctagatttgggagcacaatgaacagaggacaggaactaacttacgaatcctttgtcacaagagagtttactactactggtccgttcaatccgccttttacatttacacaaactcaagaaattctaacagtgaatgcagaaggtgttagcaccggtggtgaatattatatagatagtattgagattgttcctgtaaatccgacgcgagaggcggaagaggatctagaagcagcgaagaaagcggtggcgagcttgtttacacgtacaagggacggattacaagtaaatgtgacagattaccaagtggatcgagcggcaaatttagtgttatgcttatcagatgaacaatatgcgcatgataaaaagatgttattggaagccgtacgcgcagccaaacgactcagccgcgagcgtaacttgcttcaagatccagatttcaatgaaataaatagtacggaagatagtggttggaagacaagtaacggcattatcattagtgagggtggtccattctttaaaggtcgtgcccttcagctagcaagcgcacgtgaaaattacccaacatacatctatcaaaaggtagactcatcaatgttaaaaccttatacacgatataaactagatggatttgtgcaaagtagtcaagatttagaaattgaactcattcaccatcataaagtccacctcgtgaaaaatgtaccagataatttagtacttgatacttacccagatggttcttgcaacggaattaaccgatgtgaggaacaacagatggtgaattcgcaactagaaacagaacatcatccaatggattgctgtgaagcatcccaaacacatgagttttcttcctatattcatacaggtgacctaaatgcaagtgtagatcaaggcatttgggttgtattgaagattcggacaacagatggttctgcgacgttaggaaatcttgaattggtagaggttggtccattatcgggtgaatctctagaacgtgaacaaagagataatgcgaaatggaatgcagagttaggaaggaagcgtgcagaagcagatcgcgtgtatcaaggtgcgaaacaagcaattaaccatctatttgtagactatcaagatcaacaattaaatccagaagttgggctagcagaaattagtgaagctcgaaatcttatcgaatcaatttcagatgtatattgcgatgcagtactgcgaattcctggaattaactacgagatgtatacagagttatctaatcgtctacaacaagcagcgtatctgtatacgtctcgaaatgccgtgcaaaacggggactttaacagcggtttagatagttggaatgcaacaactgatgcgacggttcagcaggatggcaatatgtatttcttagttctttcccattgggatgcacaagtttctcaacaatttagagtacagccgaattgtaaatatgtgttacgtgtgacagcgaagaaagtagggaacggagatggatatgttacgatccaagatggcgctcatcaccgagaaacacttacattcaatgcatgtgactacgatgtaaatggtacgcatgtaaatgacaattcgtatattacaaaagaattggagttctatccaaagacagaacatatgtgggtagaggtaagtgaaacagaaggtaccttctatatagacagcattgagctaattgaaacacaagagtag

SEQ ID NO: 4 - DNA, 3540 bp, Bacillus thuringiensis
atgggaggaaaaagtatgaatcgaaataatcaaggtgaatatgaaattattgacgcttccacttgtggttgttcgtcagatgatgttgttcaatatcctttggcaagagatccgaatgctgcattccaaaatatgaattataaagattatttgaaaatgtctgacggagactacgtcgattcttatataaacccaggcttatctattggtcgtagagatgtgaccctaactggagttggtattgttgcgctaatagtagggactttaggtggtccagttgggggtatagtaactggcttgatttcctctcttttaggattattgtggccaagtaatgataatgatgtatgggaagcttttatggcacaaatagaagagctaattgaacaaaggatagcagatcaagtagtaaggaatgcactcgataacttaactggattgcgcgattattataatcaatacctattagcattggaggagtggcaggaaaggccgaacgctgtaagatctaccttagtttttaatagatttgaaaccctgcattctcactttgtaactagtatgccaagctttggtagtggccctggaagtgaaaggtatgcggtacaattgctgacagtttatgcacaagcggcaaatctgcatttgttattattaagagatgctgacatttatggggcaaggtggggacttcgtgaatctcagattgatttatattttaatgagctacaaaatcgtactcgagattataccaatcattgtgtaactgcgtacaataatgggttagaggagatacgaggaacaagccctgcaagttggttgaggtaccatcaattccgtagagagacaacactaatagcattggatttagtggcgatattcccatattacaacgtacgagaatatccaattggggtaaatcctcagcttacacgtgatgtatatacagatccaataggggttactttcagaagagaagattgggaaacaggagtagaatgcagaccatgggtaaatactccttacatgagcttttcggatcttgaaaatgcaataattcgtccaccacatctatttgaaacattacgtaatttaacaattcatacaggtcgatataacctagtaggaggggcgagatttattgaaggatgggtcggacattctgtaacaaatactcgcttgggtaattcaacagtatttacaagtaattatggttctttgccacctcgttttcaagtttttaattttactaattttgatgtttaccaaattaatacgagagcagattctacaggtacctttagaatccctggatttgcagttacaagggcccaattcattccgggtgggacttattcagtagctcaccgagatccaggggcatgtcaacaagattatgattcaattgaagagttaccaagtctagacccggatgaacctattaatagaagttatagtcatagattatcgcatgttaccctttataaatatactctctcagatacagattatggagttatcaattatacagattatggaagtatgcctgcatatgtctggacacatcgcgatgtggaccttactaacacgattactgcagatagaattacacaactcccattagtaaaggcatctacactacctgcgggtactactgtggtaaaaggcccaggatttacaggaggagatatactccgaagaacaactaatggaacatttgggacattacatgtaagggttaattcaccattaacacaacaatatcgcctaagagttcgttttgcctcaacaggaaatttcagtataagggtactccgtggagggacttctatcggtgatgctagatttgggagcacaatgaacagaggacaggaactaacttacgaatcctttgtcacaagagagtttactactactggtccgttcaatccgccttttacatttacacaaactcaagaaattctaacagtgaatgcagaaggtgttagcaccggtggtgaatattatatagatagtattgagattgttcctgtaaatccgacgcgagaggcggaagaggatctagaagcagcgaagaaagcggtggcgagcttgtttacacgtacaagggacggattacaagtaaatgtgacagattatcaagtcgatcaagcggcaaatttagtgtcatgcttatcagatgaacaatatgggtatgacaaaaagatgttattggaagcggtacgcgcggcaaaacgcctcagccgagaacgtaacttacttcaagatccagattttaatacaatcaatagtacagaagaaaatggatggaaagcaagtaacggcgttactattagtgagggcggtccattctataaaggccgtgcacttcagctagcaagtgcacgagaaaattatccaacatacatttatcaaaaagtagatgcatcggagttaaaaccttatacacgatatagactagatgggttcgtgaagagtagtcaagatttagaaattgatctcattcaccatcataaagtccatcttgtgaaaaatgtaccagataatttagtatctgatacttacccagatgattcttgtagtggaatcaatcgatgtcaggaacaacagatggtaaatgcgcaactggaaacagagcatcatcatccgatggattgctgtgaagcagctcaaacacatgagttttcttcctatattgatacaggggatttaaattcgagtgtagaccagggaatctgggcgatctttaaagttcgaacaaccgatggttatgcgacgttaggaaatcttgaattggtagaggtcggaccgttatcgggtgaatctttagaacgtgaacaaagggataatacaaaatggagtgcagagctaggaagaaagcgtgcagaaacagatcgcgtgtatcaagatgccaaacaatccatcaatcatttatttgtggattatcaagatcaacaattaaatccagaaatagggatggcagatattatggacgctcaaaatcttgtcgcatcaatttcagatgtatatagcgatgccgtactgcaaatccctggaattaactatgagatttacacagagctgtccaatcgcttacaacaagcatcgtatctgtatacgtctcgaaatgcggtgcaaaatggggactttaacaacgggctagatagctggaatgcaacagcgggtgcatcggtacaacaggatggcaatacgcatttcttagttctttctcattgggatgcacaagtttctcaacaatttagagtgcagccgaattgtaaatatgtattacgtgtaacagcagagaaagtaggcggcggagacggatacgtgactatccgggatggtgctcatcatacagaaacgcttacatttaatgcatgtgattatgatataaatggcacgtacgtgactgataatacgtatctaacaaaagaagtgatattctattcacatacagaacacatgtgggtagaggtaaatgaaacagaaggtgcatttcatatagatagtattgaattcgttgaaacagaaaagtaa

SEQ ID NO: 5 - DNA, 3444 bp, Artificial Sequence
  Synthetic Cry Gene
atggacctggatgggaataagacagagacagagaccgagattgtgaatgggagcgagagcagcattgacccgagcagcgtttcgtacgctgggaacaatagctactccagcgccctgaacctcaattcgtgccagaataggggcatcgctcagtgggttaacacgctgggcggggctattgggcaggccgtgagcatcggcacatctatcatttcactcctggccgcgccgacactcactgggtctatttcactggccttcaatctcatcaggaggatggggaccggctccaacggctcgtctatttccgacctgagcatctgcgatctcctgagcatcattaacctgcgggtttcgcaggctgtgctcaacgacgggatcgctgatttcaatggctccgttgctgtgtacgacctgtacctccacgccctgcgcagctggaacaataaccctaacgctgctactgctgaggagctgaggacccgcttcaggatcgccgattcggagttcgagaggattctgacgaggggctcgctcacacatggcggctccctcgcccgccaggacgctcaggtcctcctgctcccgtccttcgttaacgcggcttacctgcacctgctcatcctccgcgatgcttcgcgctacggggcctcttggggcctcttcaacaccacgccgcatatcaattaccccgtgaggctgcagcagctcattggcagctacacgcactactgcacacattggtacaaccaggggctgaatgagatccggcagcgcggcaacactgccgtgaattggctcgagttccaccgctaccgccgcgacatgacgctgatggtcctcgatgtggtctcgctgttctctgccctcgacacgatccgctacccgaacgctacagttgtgcagctcagccgcactgtctacaccgatccgattggcttcgttaaccgcgggtcaggcaataggctgtcctggttcgactggaggaaccaggcgaatttctctactctcgagtcagagatgccgaccccctcatccccactgagcctcaaccacatgtcgatcttcactgggcctctgaccctcccagtgtcccctaacacgcatagggcccgggtctggtacggcaaccagaatatgttcacaactgggtcacagaactccggccagaccacgaactctattcagaatatctcaggcctggagattttccgcatcgactctcaggcgtgcaatctcaataacaattcatacggcgtgaacagggcggagttcttccacggggctagccagggctcgcagcggtctgtctaccagggatacatccgccagagcggcctggacaaccctgtcgttatgaatctgcagtctttcctcccaggcgagaactcagccacccctacggcgcaggattacacccacattctgtccaacccggttaatatcaggggcgggctcaggcagattgtggccgacaggcgctcctccgtggtcgtttacggctggacgcacaagtccctgagcaggaggtcactcgtggctccagaccagatcacccaggtcccagccgttaaggcgtccccttcttcacattgcactatcattgccggcccaggcttcaccggcggggacctggtgtcgctccagcccaacggccagctcgtcatcccgttccaggtttctgcgcccgagacgaactaccacattcgcatctgctacgtctcgacgtctgattgcagcattaacacaatctgcaatgacgagacgcatctgtccacactcccgagcacaacttccagcctggagaacctccagtgcaatcacctgcattacttcaacgtgggcactttcaagccaaccatcgactcgaagctgacgctcgtcaacacatctcctaacgctaacatcattatcgacaagatcgagttcatcccggtggataccgcccagcagcagaacgaggacctcgaggccgcgaagaaggctgtcgcctccctgttcacacgcactagggacggcctccaggtcaatgttaaggactaccaggtggatcaggctgccaacctggtctcatgcctctccgacgagcagtacggctacgataagaagatgctgctcgaggccgtgagggctgctaagaggctgagcagggagaggaacctgctccaggaccccgatttcaacacaatcaactcgaccgaggagaacgggtggaaggcgtcaaatggcgtcaccatctccgagggcgggccattctacaagggcagggctattcagctcgcgtctgctcgggagaactaccccacatacatctaccagaaggtggatgcctccgagctgaagccatacacccgctaccgcctcgacggcttcgtcaagtcgtctcaggacctggagattgatctcatccaccatcacaaggtgcacctggtcaagaacgttccggacaatctcgtgagcgatacgtaccccgacgattcatgctccggaatcaacaggtgccaggagcagcagatggtcaacgcgcagctggagaccgagcatcaccatccgatggactgctgcgaggctgctcagacgcacgagttctcatcctacatcgacacaggggatctgaacagctcggtcgatcagggcatttgggccatcttcaaggttaggaccacggacgggtacgctaccctcggcaacctggagctggtggaggtcgggccactgagcggcgagtcgctcgagagggagcagagggacaacactaagtggtccgctgagctgggccgcaagagggctgagaccgaccgcgtctaccaggatgccaagcagagcatcaatcacctgttcgttgactaccaggatcagcagctcaaccccgagattggcatggcggacatcatggatgctcagaacctggtggccagcatctcggacgtgtacagcgatgcggtcctccagattccaggaatcaactacgagatctacacggagctgtcgaacaggctccagcaggcctcctacctgtacacaagccggaacgcggtccagaatggggacttcaacaatggcctcgattcatggaatgctacggctggggcttccgtgcagcaggatggcaacacacacttcctggtcctctcccattgggacgcgcaggttagccagcagttccgcgtgcagccgaactgcaagtatgtgctgagggtcactgctgagaaggttggcgggggcgacggctacgtgaccatcagggacgatgcgcaccataccgagacgctgacattcaacgcttgcgactacgacatcaacggcacctacgtgacagacaacacttacctaaccaaggaggtggtcttccacccggagactcagcatatgtgggttgaggtgaacgagaccgagggcgccttccacatagactccatcgagttcgtcgagaccgagaagtga

SEQ ID NO: 6 - DNA, 3474 bp, Artificial Sequence
  Synthetic Cry Gene
atgaacaggaacaaccagaacgagtacgagattattgacgccccccattgcggctgcccctccgacgacgatgtgaagtacccactggctagcgaccccaacgctgctctgcagaacatgaattacaaggattacctccagatgaccgacgaggattacacggactcgtacatcaacccatccctcagcatttcgggcagggacgctgtccagacagccctgactgtggtcggccgcatcctcggggcgctgggcgttcccttctcaggccagattgtgtccttctaccagttcctcctgaataccctctggccagtgaacgacacggcgatctgggaggctttcatgcgccaggtggaggagctggtcaatcagcagattacggagttcgccaggaaccaggctctcgcgcggctgcagggcctcggggactccttcaatgtctaccagaggagcctgcagaactggctcgccgaccgcaacgataccaggaatctctccgttgtgcgcgcccagttcatcgcgctcgacctggatttcgtgaatgccattcctctgttcgctgtgaacggccagcaggtcccgctcctgtccgtttacgctcaggccgtgaacctgcatctcctgctcctgaaggatgcttcgctcttcggcgaggggtggggcttcacacagggcgagatctctacttactacgaccgccagctcgagctgacagcgaggtacactaattactgcgagacctggtacaacacggggctggacaggctcaggggaaccaacacggagtcctggctccgctaccaccagttccgcagggagatgactctggtcgttctcgatgtggtcgccctgttcccatactacgacgtccgcctctacccaaccggctccaaccctcagctgacaagggaggtgtacactgaccctatcgtcttcaacccaccagctaatgtggggctctgcaggcgctggggaaccaacccgtacaatacgttcagcgagctggagaacgcgttcatccggccacctcatctgttcgatcgcctcaactctctcaccatttccagcaataggttccctgtctcgtctaacttcatggactactggtctggccacacgctgaggcggagctacctcaacgattcggctgtgcaggaggactcctacggcctcatcaccacgacacgggccaccattaacccgggggtcgatggcaccaaccggatcgagtcgacggcggtggacttccgctctgctctcatcgggatttacggcgttaacagggcttccttcgtgccaggcgggctgttcaatggcactaccagcccagctaacggcgggtgcagggacctgtacgataccaacgacgagctgccaccagacgagtccacaggctcatccactcatcgcctctcgcacgtcacattcttctctttccagactaatcaggccgggtcaatcgcgaacgctggctccgttcccacctacgtgtggacgcgcagggacgtcgatctgaacaacacgatcactccgaaccgcattacgcagctcccactggtgaaggcttctgctccagtctcaggcacgacagttctgaaggggcccggcttcaccggcgggggcatcctccggcgcactaccaatgggaccttcggcacgctgagggtgaccgtcaacagcccactgacgcagcagtacaggctccgcgtgaggttcgcttctacgggcaatttctcaatcaggctcctgagggggggcgtgagcattggggacgtcaggctgggctcgacaatgaaccggggccaggagctgacatacgagagcttcttcactcgcgagttcacgacaactggcccattcaatccacctttcaccttcacgcaggcccaggagatcctcacagttaacgctgagggcgtgtcgactgggggcgagtactacattgataggatcgagattgttccagtgaacccagctagggaggctgaggaggacctggaggctgccaagaaggctgtggccagcctgttcacacgcactagggacggcctccaggtcaatgttaccgattaccaggtcgacagggcggctaacctggtttcatgcctctccgatgagcagtactcccacgacaagaagatgctcctggaggccgtccgggctgctaagcgcctgtcacgggagcgcaacctcctgcaggaccctgatttcaacacgatcaactccactgaggagaatgggtggaaggccagcaacggcgtgaccatttcggaggggggcccgttcttcaagggccgcgcgctccagctggctagcgctagggagaactaccctacgtacatctaccagaaggtcgatgcgtcggttctgaagccgtacacacgctaccgcctcgacggcttcgtgaagtcctcccaggatctggagatcgacctcattcaccatcacaaggtccatctggttaagaacgtgcccgacaatctcgtctccgatacctacagcgacgggtcctgcagcggaatcaaccgctgcgatgagcagcagcaggtggatatgcagctcgacgccgagcatcacccaatggactgctgcgaggctgcccagacccacgagttctcttcctacatcaatacgggggatctgaacgcctccgttgaccagggcatttgggttgtgctcaaagtgaggaccacggacgggtacgctaccctgggcaacctcgagctggtggaggtcgggccgctgagcggcgagtcgctcgagagggagcagagggataacgctaagtggaatgctgagctgggcaggaagagggctgagaccgacagggtctacctggctgctaagcaggcgatcaatcacctcttcgtggattaccaggaccagcagctgaaccctgagatcggcctcgctgagattaacgaggcctctaatctggtcaagtcgatctctggggtttactcagatactctcctgcagatcccgggaattaactacgagatttacaccgagctgtccgaccggctccagcaggcttcctacctctacacgagccgcaacgccgtgcagaatggggatttcaactcgggcctggactcttggaacgcgacaactgatgcttctgtccagcaggacggctcaacccatttcctcgtgctgtcacactgggacgctcaggtgtcccagcagatgagggtcaacctgaattgcaagtacgtcctcagggttacggcgaagaaggtcgggggcggggatggctacgtcacaatcagggacggcgcgcatcaccaggagaccctcacgttcaatgcttgcgactacgatgtcaacggcacatacgttaacgacaattcctacatcactaaggaggtcgttttctaccccgagaccaagcacatgtgggttgaggtgtctgagtcggagggctcgttctacattgatagcattgagttcattgagacgcaggagtga

SEQ ID NO: 7 - DNA, 3522 bp, Artificial Sequence
  Synthetic Cry Gene
atgaaccggaacaaccagggcgagtacgagattattgatgcctccacttgcggctgctcctcagatgatgtcgtccagtacccactcgctcgcgacccgaacgctgctttccagaacatgaattacaaggactacctgaagatgtctgacggcgattacgtcgattcatacattaacccaggcctgtccatcgggaggagggacgtcacgctcacaggcgtcgggatcgttgctctcattgtgggcaccctgggcggcccagttggcgggattgtgacgggcctgatctccagcctcctggggctcctgtggccaagcaacgacaatgatgtgtgggaggccttcatggcgcagatcgaggagctgattgagcagaggatcgctgaccaggtggtccggaacgccctggacaatctcaccggcctgagggattactacaaccagtacctcctggctctcgaggagtggcaggagaggcccaatgccgtgaggtctacgctggtcttcaaccggttcgagacgctccattcacacttcgtgacatcaatgccatccttcggcagcgggcctggcagcgagcgctacgcggttcagctcctgaccgtgtacgctcaggctgccaacctgcacctcctgctcctgagggacgctgatatctacggcgctcggtgggggctcagggagtcccagatcgacctctacttcaacgagctgcagaatcggacgcgcgattacacaaaccattgcgtcacagcctacaacaatggcctggaggagatcagggggacttcgccagcttcttggctgcgctaccaccagttccggcgcgagaccacgctcattgccctcgacctggtggcgatcttcccatactacaatgtcagggagtacccaattggcgttaaccctcagctcacgcgggacgtgtacacagatccgatcggcgtcacgttcaggcgggaggactgggagacaggcgtcgagtgcaggccgtgggttaataccccatacatgtctttctcagatctggagaacgccatcattaggccgccccatctcttcgagacgctccggaatctgacgattcacacaggcaggtacaacctggtcggcggggcgaggttcatcgagggctgggtcgggcattccgttactaataccaggctgggcaacagcactgtgttcaccagcaattacgggtcgctcccacctcggttccaggtgttcaacttcacgaatttcgacgtctaccagatcaacacacgggccgattcgacgggcacattccgcattccggggttcgcggtcactagggctcagttcatccccggcgggacctactccgtggctcaccgcgacccaggcgcttgccagcaggactacgattcaattgaggagctgccctccctggacccagatgagcctatcaaccggtcctacagccatcgcctctcacacgtcaccctgtacaagtacactctctccgacaccgattacggcgtgatcaattacaccgactacgggagcatgccagcttacgtgtggacgcatcgcgacgtcgatctgactaacaccattacggcggataggatcacgcagctcccgctggtgaaggcttcgacactccccgccggcacaactgttgtgaaggggcccggcttcaccggcggggacatcctgaggaggaccacgaatggcacgttcgggacactccacgtgagggtcaacagcccactgacccagcagtacaggctccgggtccgcttcgcttcgacgggcaacttctctattagggtgctgaggggcgggacatctatcggcgacgctcgcttcgggtcaactatgaacaggggccaggagctgacttacgagtccttcgtgacccgcgagttcacaactaccggcccgttcaatccgcccttcacattcactcagacccaggagatcctgactgtcaacgctgagggcgtttcgaccggcggggagtactacatcgactctattgagatcgttccagtgaacccaaccagggaggctgaggaggatctcgaggctgctaagaaggccgtcgcgagcctgttcacgaggacacgggacggcctccaggtcaatgttacggactaccaggttgatagggctgctaacctcgtgctgtgcctctccgacgagcagtacgcccacgataagaagatgctcctggaggcggtgagggctgctaagaggctgagcagggagaggaacctcctgcaggaccctgatttcaacgagatcaattctactgaggactcaggctggaagaccagcaacgggatcattatctcggagggcgggccgttcttcaagggccgggccctgcagctcgcttccgctcgcgagaactaccctacctacatctaccagaaggtggactcgtctatgctgaagccgtacacgaggtacaagctcgacggcttcgtgcagtcatcccaggatctcgagattgagctgatccaccatcacaaggtgcacctcgtcaagaacgttccagacaatctggtcctcgacacctaccctgatggctcgtgcaacggaatcaaccgctgcgaggagcagcagatggtgaactctcagctggagacggagcatcaccctatggactgctgcgaggcctcacagactcatgagttcagctcgtacatccacaccggcgacctcaacgcgtctgtcgatcaggggatttgggtcgttctgaagatcaggacgacagacggctcggctaccctcgggaacctggagctggtggaggtcggccccctgtcaggggagtccctcgagagggagcagagggacaacgccaagtggaatgctgagctgggccggaagcgcgctgaggctgatcgcgtgtaccagggcgctaagcaggccatcaatcacctcttcgtcgactaccaggatcagcagctgaaccctgaggttggcctcgcggagatcagcgaggctcggaacctgattgagtcgatctctgacgtgtactgcgatgccgtcctccgcattccgggaatcaactacgagatgtacacggagctgtccaacaggctgcagcaggctgcttacctgtacacaagccgcaacgcggtgcagaatggcgacttcaactccgggctcgatagctggaatgctactaccgacgccaccgttcagcaggatggcaacatgtacttcctggtgctcagccactgggacgcccaggtttcgcagcagttccgcgtgcagccaaattgcaagtatgtgctgagggtcacagcgaagaaggtcgggaacggcgacggctacgtgactatccaggatggcgcgcatcaccgcgagactctgaccttcaatgcttgcgactacgatgttaacggcacgcatgtgaacgacaattcctacattacaaaggagctggagttctacccgaagactgagcacatgtgggttgaggtgagcgagactgagggcaccttctacatagattcgatcgagctgattgagacccaggagtga

SEQ ID NO: 8 - DNA, 3540 bp, Artificial Sequence
  Synthetic Cry Gene
atgggggggaagtctatgaacaggaacaaccagggcgagtacgagattattgatgcctccacatgcgggtgctccagcgacgacgtggtccagtacccactcgctcgcgaccctaacgctgctttccagaacatgaattacaaggactacctgaagatgtccgacggcgattacgtggatagctacattaacccaggcctctcgatcgggaggagggacgtcactctgaccggggttggcatcgtggcgctgattgttggcacactcggcgggcctgtgggcgggattgtcactggcctcatctccagcctcctggggctcctgtggccatccaacgacaatgatgtctgggaggcgttcatggctcagatcgaggagctgattgagcagcgcatcgcggaccaggtggtcaggaacgctctcgacaatctgaccggcctcagggattactacaaccagtacctcctggctctcgaggagtggcaggagaggccaaatgccgtgcgctccacgctcgttttcaaccgcttcgagaccctgcacagccatttcgtgacgagcatgccgtcgttcgggtctggccccgggtcggagcgctacgctgtgcagctcctgaccgtctacgcccaggctgccaacctccacctcctgctcctgcgcgacgctgatatctacggcgccaggtgggggctcagggagagccagatcgacctgtacttcaacgagctgcagaatcggacacgcgattacactaaccactgcgtcaccgcctacaacaatggcctcgaggagatcagggggacgtcaccagcttcctggctccgctaccaccagttccggagggagaccacgctgattgcgctcgacctggtggctatcttcccctactacaatgtgcgcgagtacccgattggcgtcaacccccagctgaccagggacgtttacaccgacccgatcggcgtgacattcaggcgggaggactgggagactggcgtggagtgcaggccgtgggtcaataccccatacatgtctttctcagacctcgagaacgccatcattaggccgccccacctgttcgagacgctgaggaatctcaccattcatacgggcaggtacaacctggtcggcggggcgcgcttcatcgagggctgggttgggcactcagtgacgaacacaaggctcggcaattccacagtgttcacttccaactacggcagcctgccacctcggttccaggttttcaacttcacaaatttcgacgtgtaccagatcaacactagggccgattcgactggcaccttccggattccagggttcgccgttacccgcgcgcagttcatccctggcgggacgtactccgtggctcaccgcgacccgggcgcttgccagcaggactacgatagcattgaggagctgccctcgctcgacccagatgagcctatcaacaggtcctacagccaccggctgtctcatgtcaccctctacaagtacaccctgtcagacacggattacggcgtgatcaattacaccgactacgggtccatgccagcttacgtttggacgcaccgggacgtggatctcacgaacacaattactgccgaccgcatcacacagctcccactggtgaaggccagcactctgcctgcgggcacaactgttgtgaagggccctgggttcaccggcggggacatcctcaggaggaccacgaatggcaccttcgggacgctgcatgtccgcgttaactccccgctcacacagcagtacaggctgcgggtgcgcttcgcttcgactggcaacttctctattcgcgtcctcaggggcgggacctccatcggcgacgctaggttcgggagcacgatgaacaggggccaggagctgacatacgagtccttcgtcactagggagttcacaactaccggcccgttcaatccgcccttcaccttcacgcagacacaggagattctcaccgttaacgctgagggcgtgagcacgggcggggagtactacatcgactcgatcgagattgtgccagtcaacccaaccagggaggctgaggaggatctggaggctgctaagaaggccgtggcgagcctcttcactaggacccgggacggcctgcaggttaatgtgacggactaccaggtcgatcaggccgcgaacctggttagctgcctctcggacgagcagtacggctacgataagaagatgctcctggaggccgtccgcgctgctaagaggctctcgagggagaggaacctcctgcaggaccccgatttcaacacaattaattctactgaggagaacggctggaaggcctctaatggggtgaccatctcagagggcgggccattctacaagggcagggcgctccagctggcttcagctcgggagaactaccccacctacatctaccagaaggtcgacgcctccgagctgaagccatacacgcgctaccgcctggatggcttcgtgaagtcgtctcaggacctggagatcgatctcattcaccatcacaaggtccacctcgttaagaacgtgccggacaatctggtctccgatacctaccccgacgattcgtgctctggaatcaacaggtgccaggagcagcagatggtgaacgcccagctcgagacggagcatcaccatcctatggactgctgcgaggcggctcagacccatgagttctcatcctacatcgacacgggcgatctcaacagctcggtcgaccaggggatctgggcgattttcaaggttaggacgacagatggctacgctaccctggggaatctcgagctggtcgaggttggccccctctctggggagtcactggagagggagcagagggacaacacaaagtggtctgctgagctgggcaggaagcgggctgagactgaccgcgtctaccaggatgccaagcagtccatcaatcacctcttcgtggactaccaggatcagcagctgaaccctgagattggcatggctgacatcatggatgcccagaacctcgtcgcgtcaatctccgacgtctacagcgatgcggttctgcagatcccgggcattaattacgagatctacacagagctgtcgaacaggctccagcaggcgtcatacctctacacgtcccggaacgctgtgcagaatggcgacttcaacaatgggctggattcgtggaatgcgacagctggcgcctctgtgcagcaggacgggaacactcacttcctcgtcctgtctcattgggatgcccaggtctcacagcagttccgggttcagccgaactgcaagtatgtgctgcgcgttaccgctgagaaagtgggcgggggcgacggctacgtcacgatccgcgatggggctcaccatacggagacactcactttcaacgcctgcgactacgatatcaatggcacatacgttactgacaacacctacctgacgaaggaggtcatcttctactcccacacagagcatatgtgggtggaggtcaacgagactgagggcgccttccacatcgacagcattgagttcgtggagaccgagaagtga

SEQ ID NO: 9 - DNA, 3444 bp, Artificial Sequence
  Synthetic Cry Gene
atggacctggatgggaataagacagagacagagaccgagattgtgaatgggagcgagagcagcattgacccgagcagcgtttcgtacgctgggaacaatagctactccagcgccctgaacctcaattcgtgccagaataggggcatcgctcagtgggttaacacgctgggcggggctattgggcaggccgtgagcatcggcacatctatcatttcactcctggccgcgccgacactcactgggtctatttcactggccttcaatctcatcaggaggatggggaccggctccaacggctcgtctatttccgacctgagcatctgcgatctcctgagcatcattaacctgcgggtttcgcaggctgtgctcaacgacgggatcgctgatttcaatggctccgttgctgtgtacgacctgtacctccacgccctgcgcagctggaacaataaccctaacgctgctactgctgaggagctgaggacccgcttcaggatcgccgattcggagttcgagaggattctgacgaggggctcgctcacacatggcggctccctcgcccgccaggacgctcaggtcctcctgctcccgtccttcgttaacgcggcttacctgcacctgctcatcctccgcgatgcttcgcgctacggggcctcttggggcctcttcaacaccacgccgcatatcaattaccccgtgaggctgcagcagctcattggcagctacacgcactactgcacacattggtacaaccaggggctgaatgagatccggcagcgcggcaacactgccgtgaattggctcgagttccaccgctaccgccgcgacatgacgctgatggtcctcgatgtggtctcgctgttctctgccctcgacacgatccgctacccgaacgctacagttgtgcagctcagccgcactgtctacaccgatccgattggcttcgttaaccgcgggtcaggcaataggctgtcctggttcgactggaggaaccaggcgaatttctctactctcgagtcagagatgccgaccccctcatccccactgagcctcaaccacatgtcgatcttcactgggcctctgaccctcccagtgtcccctaacacgcatagggcccgggtctggtacggcaaccagaatatgttcacaactgggtcacagaactccggccagaccacgaactctattcagaatatctcaggcctggagattttccgcatcgactctcaggcgtgcaatctcaataacaattcatacggcgtgaacagggcggagttcttccacggggctagccagggctcgcagcggtctgtctaccagggatacatccgccagagcggcctggacaaccctgtcgttatgaatctgcagtctttcctcccaggcgagaactcagccacccctacggcgcaggattacacccacattctgtccaacccggttaatatcaggggcgggctcaggcagattgtggccgacaggcgctcctccgtggtcgtttacggctggacgcacaagtccctgagcaggaggtcactcgtggctccagaccagatcacccaggtcccagccgttaaggcgtccccttcttcacattgcactatcattgccggcccaggcttcaccggcggggacctggtgtcgctccagcccaacggccagctcgtcatcccgttccaggtttctgcgcccgagacgaactaccacattcgcatctgctacgtctcgacgtctgattgcagcattaacacaatctgcaatgacgagacgcatctgtccacactcccgagcacaacttccagcctggagaacctccagtgcaatcacctgcattacttcaacgtgggcactttcaagccaaccatcgactcgaagctgacgctcgtcaacacatctcctaacgctaacatcattatcgacaagatcgagttcatcccggtggataccgcccagcagcagaacgaggacctcgaggccgcgaagaaggctgtcgcctccctgttcacacgcactagggacggcctccaggtcaatgttaaggactaccaggtggatcaggctgccaacctggtctcatgcctctccgacgagcagtacggctacgataagaagatgctgctcgaggccgtgagggctgctaagaggctgagcagggagaggaacctgctccaggaccccgatttcaacacaatcaactcgaccgaggagaacgggtggaaggcgtcaaatggcgtcaccatctccgagggcgggccattctacaagggcagggctattcagctcgcgtctgctcgggagaactaccccacatacatctaccagaaggtggatgcctccgagctgaagccatacacccgctaccgcctcgacggcttcgtcaagtcgtctcaggacctggagattgatctcatccaccatcacaaggtgcacctggtcaagaacgttccggacaatctcgtgagcgatacgtaccccgacgattcatgctccggaatcaacaggtgccaggagcagcagatggtcaacgcgcagctggagaccgagcatcaccatccgatggactgctgcgaggctgctcagacgcacgagttctcatcctacatcgacacaggggatctgaacagctcggtcgatcagggcatttgggccatcttcaaggttaggaccacggacgggtacgctaccctcggcaacctggagctggtggaggtcgggccactgagcggcgagtcgctcgagagggagcagagggacaacactaagtggtccgctgagctgggccgcaagagggctgagaccgaccgcgtctaccaggatgccaagcagagcatcaatcacctgttcgttgactaccaggatcagcagctcaaccccgagattggcatggcggacatcatggatgctcagaacctggtggccagcatctcggacgtgtacagcgatgcggtcctccagattccaggaatcaactacgagatctacacggagctgtcgaacaggctccagcaggcctcctacctgtacacaagccggaacgcggtccagaatggggacttcaacaatggcctcgattcatggaatgctacggctggggcttccgtgcagcaggatggcaacacacacttcctggtcctctcccattgggacgcgcaggttagccagcagttccgcgtgcagccgaactgcaagtatgtgctgagggtcactgctgagaaggttggcgggggcgacggctacgtgaccatcagggacgatgcgcaccataccgagacgctgacattcaacgcttgcgactacgacatcaacggcacctacgtgacagacaacacttacatcaccaaggaggtggtcttccacccggagactcagcatatgtgggttgaggtgaacgagaccgagggcgccttccaccttgactccatcgagttcgtcgagaccgagaagtga

SEQ ID NO: 10 - DNA, 3474 bp, Artificial Sequence
  Synthetic Cry Gene
atgaacaggaacaaccagaacgagtacgagattattgacgccccccattgcggctgcccctccgacgacgatgtgaagtacccactggctagcgaccccaacgctgctctgcagaacatgaattacaaggattacctccagatgaccgacgaggattacacggactcgtacatcaacccatccctcagcatttcgggcagggacgctgtccagacagccctgactgtggtcggccgcatcctcggggcgctgggcgttcccttctcaggccagattgtgtccttctaccagttcctcctgaataccctctggccagtgaacgacacggcgatctgggaggctttcatgcgccaggtggaggagctggtcaatcagcagattacggagttcgccaggaaccaggctctcgcgcggctgcagggcctcggggactccttcaatgtctaccagaggagcctgcagaactggctcgccgaccgcaacgataccaggaatctctccgttgtgcgcgcccagttcatcgcgctcgacctggatttcgtgaatgccattcctctgttcgctgtgaacggccagcaggtcccgctcctgtccgtttacgctcaggccgtgaacctgcatctcctgctcctgaaggatgcttcgctcttcggcgaggggtggggcttcacacagggcgagatctctactcactacgaccgccagctcgagctgacagcgaggtacactaattactgcgagacctggtacaacacggggctggacaggctcaggggaaccaacacggagtcctggctccgctaccaccagttccgcagggagatgactctggtcgttctcgatgtggtcgccctgttcccatactacgacgtccgcctctacccaaccggctccaaccctcagctgacaagggaggtgtacactgaccctatcgtcttcaacccaccagctaatgtggggctctgcaggcgctggggaaccaacccgtacaatacgttcagcgagctggagaacgcgttcatccggccacctcatctgttcgatcgcatccagtctctctcaatttccagcaataggttccctgtctcgtctaacttcatggactactggtctggccacacgctgaggcggagctacctcaacgattcggctgtgcaggaggactcctacggcctcatcaccacgacacgggccaccattaacccgggggtcgatggcaccaaccggatcgagtcgacggcggtggacttccgctctgctctcatcgggatttacggcgttaacagggcttccttcgtgccaggcgggctgttcaatggcactaccagcccagctaacggcgggtgcagggacctgtacgataccaacgacgagctgccaccagacgagtccacaggctcatccactcatcgcctctcgcacgtcacattcttctctttccagactaatcaggccgggtcaatcgcgaacgctggctccgttcccacctacgtgtggacgcgcagggacgtcgatctgaacaacacgatcactccgaaccgcattacgcagctcccactggtgaaggcttctgctccagtctcaggcacgacagttctgaaggggcccggcttcaccggcgggggcatcctccggcgcactaccaatgggaccttcggcacgctgagggtgaccgtcaacagcccactgacgcagcagtacaggctccgcgtgaggttcgcttctacgggcaatttctcaatcaggctcctgagggggggcgtgagcattggggacgtcaggctgggctcgacaatgaaccggggccaggagctgacatacgagagcttcttcactcgcgagttcacgacaactggcccattcaatccacctttcaccttcacgcaggcccaggagatcctcacagttaacgctgagggcgtgtcgactgggggcgagtactacattgataggatcgagattgttccagtgaacccagctagggaggctgaggaggacctggaggctgccaagaaggctgtggccagcctgttcacacgcactagggacggcctccaggtcaatgttaccgattaccaggtcgacagggcggctaacctggtttcatgcctctccgatgagcagtactcccacgacaagaagatgctcctggaggccgtccgggctgctaagcgcctgtcacgggagcgcaacctcctgcaggaccctgatttcaacacgatcaactccactgaggagaatgggtggaaggccagcaacggcgtgaccatttcggaggggggcccgttcttcaagggccgcgcgctccagctggctagcgctagggagaactaccctacgtacatctaccagaaggtcgatgcgtcggttctgaagccgtacacacgctaccgcctcgacggcttcgtgaagtcctcccaggatctggagatcgacctcattcaccatcacaaggtccatctggttaagaacgtgcccgacaatctcgtctccgatacctacagcgacgggtcctgcagcggaatcaaccgctgcgatgagcagcagcaggtggatatgcagctcgacgccgagcatcacccaatggactgctgcgaggctgcccagacccacgagttctcttcctacatcaatacgggggatctgaacgcctccgttgaccagggcatttgggttgtgctcaaagtgaggaccacggacgggtacgctaccctgggcaacctcgagctggtggaggtcgggccgctgagcggcgagtcgctcgagagggagcagagggataacgctaagtggaatgctgagctgggcaggaagagggctgagaccgacagggtctacctggctgctaagcaggcgatcaatcacctcttcgtggattaccaggaccagcagctgaaccctgagatcggcctcgctgagattaacgaggcctctaatctggtcaagtcgatctctggggtttactcagatactctcctgcagatcccgggaattaactacgagatttacaccgagctgtccgaccggctccagcaggcttcctacctctacacgagccgcaacgccgtgcagaatggggatttcaactcgggcctggactcttggaacgcgacaactgatgcttctgtccagcaggacggctcaacccatttcctcgtgctgtcacactgggacgctcaggtgtcccagcagatgagggtcaacctgaattgcaagtacgtcctcagggttacggcgaagaaggtcgggggcggggatggctacgtcacaatcagggacggcgcgcatcaccaggagaccctcacgttcaatgcttgcgactacgatgtcaacggcacatacgttaacgacaattcctacatcactaaggaggtcgttttctaccccgagaccaagcacatgtgggttgaggtgtctgagtcggagggctcgttctacattgatagcattgagttcattgagacgcaggagtga

SEQ ID NO: 11 - DNA, 3522 bp, Artificial Sequence
  Synthetic Cry Gene
atgaaccggaacaaccagggcgagtacgagattattgatgcctccacttgcggctgctcctcagatgatgtcgtccagtacccactcgctcgcgacccgaacgctgctttccagaacatgaattacaaggactacctgaagatgtctgacggcgattacgtcgattcatacattaacccaggcctgtccatcgggaggagggacgtcacgctcacaggcgtcgggatcgttgctctcattgtgggcaccctgggcggcccagttggcgggattgtgacgggcctgatctccagcctcctggggctcctgtggccaagcaacgacaatgatgtgtgggaggccttcatggcgcagatcgaggagctgattgagcagaggatcgctgaccaggtggtccggaacgccctggacaatctcaccggcctgagggattactacaaccagtacctcctggctctcgaggagtggcaggagaggcccaatgccgtgaggtctacgctggtcttcaaccggttcgagacgctccattcacacttcgtgacatcaatgccatccttcggcagcgggcctggcagcgagcgctacgcggttcagctcctgaccgtgtacgctcaggctgccaacctgcacctcctgctcctgagggacgctgatatctacggcgctcggtgggggctcagggagtcccagatcgacctctacttcaacgagctgcagaatcggacgcgcgattacacaaaccattgcgtcacagcctacaacaatggcctggaggagatcagggggacttcgccagcttcttggctgcgctaccaccagttccggcgcgagaccacgctcattgccctcgacctggtggcgatcttcccatactacaatgtcagggagtacccaattggcgttaaccctcagctcacgcgggacgtgtacacagatccgatcggcgtcacgttcaggcgggaggactgggagacaggcgtcgagtgcaggccgtgggttaataccccatacatgtctttctcagatctggagaacgccatcattaggccgccccatctcttcgagacgctccggaatctgacgattcacacaggcaggtacaacctggtcggcggggcgaggttcatcgagggctgggtcgggcattccgttactaataccaggctgggcaacagcactgtgttcaccagcaattacgggtcgctcccacctcggttccaggtgttcaacttcacgaatttcgacgtctaccagatcaacacacgggccgattcgacgggcacattccgcattccggggttcgcggtcactagggctcagttcatccccggcgggacctactccgtggctcaccgcgacccaggcgcttgccagcaggactacgattcaattgaggagctgccctccctggacccagatgagcctatcaaccggtcctacagccatcgcctctcacacgtcaccctgtacaagtacactctctccgacaccgattacggcgtgatcaattacaccgactacgggagcatgccagcttacgtgtggacgcatcgcgacgtcgatctgactaacaccattacggcggataggatcacgcagctcccgctggtgaaggcttcgacactccccgccggcacaactgttgtgaaggggcccggcttcaccggcggggacatcctgaggaggaccacgaatggcacgttcgggacactccacgtgagggtcaacagcccactgacccagcagtacaggctccgggtccgcttcgcttcgacgggcaacttctctattagggtgctgaggggcgggacatctatcggcgacgctcgcttcgggtcaactatgaacaggggccaggagctgacttacgagtccttcgtgacccgcgagttcacaactaccggcccgttcaatccgcccttcacattcactcagacccaggagatcctgactgtcaacgctgagggcgtttcgaccggcggggagtactacatcgactctattgagatcgttccagtgaacccaaccagggaggctgaggaggatctcgaggctgctaagaaggccgtcgcgagcctgttcacgaggacacgggacggcctccaggtcaatgttacggactaccaggttgatagggctgctaacctcgtgctgtgcctctccgacgagcagtacgcccacgataagaagatgctcctggaggcggtgagggctgctaagaggctgagcagggagaggaacctcctgcaggaccctgatttcaacgagatcaattctactgaggactcaggctggaagaccagcaacgggatcattatctcggagggcgggccgttcttcaagggccgggccctgcagctcgcttccgctcgcgagaactaccctacctacatctaccagaaggtggactcgtctatgctgaagccgtacacgaggtacaagctcgacggcttcgtgcagtcatcccaggatctcgagattgagctgatccaccatcacaaggtgcacctcgtcaagaacgttccagacaatctggtcctcgacacctaccctgatggctcgtgcaacggaatcaaccgctgcgaggagcagcagatggtgaactctcagctggagacggagcatcaccctatggactgctgcgaggcctcacagactcatgagttcagctcgtacatccacaccggcgacctcaacgcgtctgtcgatcaggggatttgggtcgttctgaagatcaggacgacagacggctcggctaccctcgggaacctggagctggtggaggtcggccccctgtcaggggagtccctcgagagggagcagagggacaacgccaagtggaatgctgagctgggccggaagcgcgctgaggctgatcgcgtgtaccagggcgctaagcaggccatcaatcacctcttcgtcgactaccaggatcagcagctgaaccctgaggttggcctcgcggagatcagcgaggctcggaacctgattgagtcgatctctgacgtgtactgcgatgccgtcctccgcattccgggaatcaactacgagatgtacacggagctgtccaacaggctgcagcaggctgcttacctgtacacaagccgcaacgcggtgcagaatggcgacttcaactccgggctcgatagctggaatgctactaccgacgccaccgttcagcaggatggcaacatgtacttcctggtgctcagccactgggacgcccaggtttcgcagcagttccgcgtgcagccaaattgcaagtatgtgctgagggtcacagcgaagaaggtcgggaacggcgacggctacgtgactatccaggatggcgcgcatcaccgcgagactctgaccttcaatgcttgcgactacgatgttaacggcacgcatgtgaacgacaattcctacctcacaaaggagctggagttctacccgaagactgagcacatgtgggttgaggtgagcgagactgagggcaccttctaccttgattcgatcgagctgattgagacccaggagtga

SEQ ID NO: 12 - DNA, 3540 bp, Artificial Sequence
  Synthetic Cry Gene
atgggggggaagtctatgaacaggaacaaccagggcgagtacgagattattgatgcctccacatgcgggtgctccagcgacgacgtggtccagtacccactcgctcgcgaccctaacgctgctttccagaacatgaattacaaggactacctgaagatgtccgacggcgattacgtggatagctacattaacccaggcctctcgatcgggaggagggacgtcactctgaccggggttggcatcgtggcgctgattgttggcacactcggcgggcctgtgggcgggattgtcactggcctcatctccagcctcctggggctcctgtggccatccaacgacaatgatgtctgggaggcgttcatggctcagatcgaggagctgattgagcagcgcatcgcggaccaggtggtcaggaacgctctcgacaatctgaccggcctcagggattactacaaccagtacctcctggctctcgaggagtggcaggagaggccaaatgccgtgcgctccacgctcgttttcaaccgcttcgagaccctgcacagccatttcgtgacgagcatgccgtcgttcgggtctggccccgggtcggagcgctacgctgtgcagctcctgaccgtctacgcccaggctgccaacctccacctcctgctcctgcgcgacgctgatatctacggcgccaggtgggggctcagggagagccagatcgacctgtacttcaacgagctgcagaatcggacacgcgattacactaaccactgcgtcaccgcctacaacaatggcctcgaggagatcagggggacgtcaccagcttcctggctccgctaccaccagttccggagggagaccacgctgattgcgctcgacctggtggctatcttcccctactacaatgtgcgcgagtacccgattggcgtcaacccccagctgaccagggacgtttacaccgacccgatcggcgtgacattcaggcgggaggactgggagactggcgtggagtgcaggccgtgggtcaataccccatacatgtctttctcagacctcgagaacgccatcattaggccgccccacctgttcgagacgctgaggaatctcaccattcatacgggcaggtacaacctggtcggcggggcgcgcttcatcgagggctgggttgggcactcagtgacgaacacaaggctcggcaattccacagtgttcacttccaactacggcagcctgccacctcggttccaggttttcaacttcacaaatttcgacgtgtaccagatcaacactagggccgattcgactggcaccttccggattccagggttcgccgttacccgcgcgcagttcatccctggcgggacgtactccgtggctcaccgcgacccgggcgcttgccagcaggactacgatagcattgaggagctgccctcgctcgacccagatgagcctatcaacaggtcctacagccaccggctgtctcatgtcaccctctacaagtacaccctgtcagacacggattacggcgtgatcaattacaccgactacgggtccatgccagcttacgtttggacgcaccgggacgtggatctcacgaacacaattactgccgaccgcatcacacagctcccactggtgaaggccagcactctgcctgcgggcacaactgttgtgaagggccctgggttcaccggcggggacatcctcaggaggaccacgaatggcaccttcgggacgctgcatgtccgcgttaactccccgctcacacagcagtacaggctgcgggtgcgcttcgcttcgactggcaacttctctattcgcgtcctcaggggcgggacctccatcggcgacgctaggttcgggagcacgatgaacaggggccaggagctgacatacgagtccttcgtcactagggagttcacaactaccggcccgttcaatccgcccttcaccttcacgcagacacaggagattctcaccgttaacgctgagggcgtgagcacgggcggggagtactacatcgactcgatcgagattgtgccagtcaacccaaccagggaggctgaggaggatctggaggctgctaagaaggccgtggcgagcctcttcactaggacccgggacggcctgcaggttaatgtgacggactaccaggtcgatcaggccgcgaacctggttagctgcctctcggacgagcagtacggctacgataagaagatgctcctggaggccgtccgcgctgctaagaggctctcgagggagaggaacctcctgcaggaccccgatttcaacacaattaattctactgaggagaacggctggaaggcctctaatggggtgaccatctcagagggcgggccattctacaagggcagggcgctccagctggcttcagctcgggagaactaccccacctacatctaccagaaggtcgacgcctccgagctgaagccatacacgcgctaccgcctggatggcttcgtgaagtcgtctcaggacctggagatcgatctcattcaccatcacaaggtccacctcgttaagaacgtgccggacaatctggtctccgatacctaccccgacgattcgtgctctggaatcaacaggtgccaggagcagcagatggtgaacgcccagctcgagacggagcatcaccatcctatggactgctgcgaggcggctcagacccatgagttctcatcctacatcgacacgggcgatctcaacagctcggtcgaccaggggatctgggcgattttcaaggttaggacgacagatggctacgctaccctggggaatctcgagctggtcgaggttggccccctctctggggagtcactggagagggagcagagggacaacacaaagtggtctgctgagctgggcaggaagcgggctgagactgaccgcgtctaccaggatgccaagcagtccatcaatcacctcttcgtggactaccaggatcagcagctgaaccctgagattggcatggctgacatcatggatgcccagaacctcgtcgcgtcaatctccgacgtctacagcgatgcggttctgcagatcccgggcattaattacgagatctacacagagctgtcgaacaggctccagcaggcgtcatacctctacacgtcccggaacgctgtgcagaatggcgacttcaacaatgggctggattcgtggaatgcgacagctggcgcctctgtgcagcaggacgggaacactcacttcctcgtcctgtctcattgggatgcccaggtctcacagcagttccgggttcagccgaactgcaagtatgtgctgcgcgttaccgctgagaaagtgggcgggggcgacggctacgtcacgatccgcgatggggctcaccatacggagacactcactttcaacgcctgcgactacgatatcaatggcacatacgttactgacaacacctacctgacgaaggaggtcatcttctactcccacacagagcatatgtgggtggaggtcaacgagactgagggcgccttccacctcgacagccttgagttcgtggagaccgagaagtga

SEQ ID NO: 13 - protein, 1147 aa, Bacillus thuringiensis
MDLDGNKTETETEIVNGSESSIDPSSVSYAGNNSYSSALNLNSCQNRGIAQWVNTLGGAIGQAVSIGTSIISLLAAPTLTGSISLAFNLIRRMGTGSNGSSISDLSICDLLSIINLRVSQAVLNDGIADFNGSVAVYDLYLHALRSWNNNPNAATAEELRTRFRIADSEFERILTRGSLTHGGSLARQDAQVLLLPSFVNAAYLHLLILRDASRYGASWGLFNTTPHINYPVRLQQLIGSYTHYCTHWYNQGLNEIRQRGNTAVNWLEFHRYRRDMTLMVLDVVSLFSALDTIRYPNATVVQLSRTVYTDPIGFVNRGSGNRLSWFDWRNQANFSTLESEMPTPSSPLSLNHMSIFTGPLTLPVSPNTHRARVWYGNQNMFTTGSQNSGQTTNSIQNISGLEIFRIDSQACNLNNNSYGVNRAEFFHGASQGSQRSVYQGYIRQSGLDNPVVMNLQSFLPGENSATPTAQDYTHILSNPVNIRGGLRQIVADRRSSVVVYGWTHKSLSRRSLVAPDQITQVPAVKASPSSHCTIIAGPGFTGGDLVSLQPNGQLVIPFQVSAPETNYHIRICYVSTSDCSINTICNDETHLSTLPSTTSSLENLQCNHLHYFNVGTFKPTIDSKLTLVNTSPNANIIIDKIEFIPVDTAQQQNEDLEAAKKAVASLFTRTRDGLQVNVKDYQVDQAANLVSCLSDEQYGYDKKMLLEAVRAAKRLSRERNLLQDPDFNTINSTEENGWKASNGVTISEGGPFYKGRAIQLASARENYPTYIYQKVDASELKPYTRYRLDGFVKSSQDLEIDLIHHHKVHLVKNVPDNLVSDTYPDDSCSGINRCQEQQMVNAQLETEHHHPMDCCEAAQTHEFSSYIDTGDLNSSVDQGIWAIFKVRTTDGYATLGNLELVEVGPLSGESLEREQRDNTKWSAELGRKRAETDRVYQDAKQSINHLFVDYQDQQLNPEIGMADIMDAQNLVASISDVYSDAVLQIPGINYEIYTELSNRLQQASYLYTSRNAVQNGDFNNGLDSWNATAGASVQQDGNTHFLVLSHWDAQVSQQFRVQPNCKYVLRVTAEKVGGGDGYVTIRDDAHHTETLTFNACDYDINGTYVTDNTYLTKEVVFHPETQHMWVEVNETEGAFHIDSIEFVETEK

SEQ ID NO: 14 - protein, 1157 aa, Bacillus thuringiensis
MNRNNQNEYEIIDAPHCGCPSDDDVKYPLASDPNAALQNMNYKDYLQMTDEDYTDSYINPSLSISGRDAVQTALTVVGRILGALGVPFSGQIVSFYQFLLNTLWPVNDTAIWEAFMRQVEELVNQQITEFARNQALARLQGLGDSFNVYQRSLQNWLADRNDTRNLSVVRAQFIALDLDFVNAIPLFAVNGQQVPLLSVYAQAVNLHLLLLKDASLFGEGWGFTQGEISTYYDRQLELTARYTNYCETWYNTGLDRLRGTNTESWLRYHQFRREMTLVVLDVVALFPYYDVRLYPTGSNPQLTREVYTDPIVFNPPANVGLCRRWGTNPYNTFSELENAFIRPPHLFDRLNSLTISSNRFPVSSNFMDYWSGHTLRRSYLNDSAVQEDSYGLITTTRATINPGVDGTNRIESTAVDFRSALIGIYGVNRASFVPGGLFNGTTSPANGGCRDLYDTNDELPPDESTGSSTHRLSHVTFFSFQTNQAGSIANAGSVPTYVWTRRDVDLNNTITPNRITQLPLVKASAPVSGTTVLKGPGFTGGGILRRTTNGTFGTLRVTVNSPLTQQYRLRVRFASTGNFSIRLLRGGVSIGDVRLGSTMNRGQELTYESFFTREFTTTGPFNPPFTFTQAQEILTVNAEGVSTGGEYYIDRIEIVPVNPAREAEEDLEAAKKAVASLFTRTRDGLQVNVTDYQVDRAANLVSCLSDEQYSHDKKMLLEAVRAAKRLSRERNLLQDPDFNTINSTEENGWKASNGVTISEGGPFFKGRALQLASARENYPTYIYQKVDASVLKPYTRYRLDGFVKSSQDLEIDLIHHHKVHLVKNVPDNLVSDTYSDGSCSGINRCDEQQQVDMQLDAEHHPMDCCEAAQTHEFSSYINTGDLNASVDQGIWVVLKVRTTDGYATLGNLELVEVGPLSGESLEREQRDNAKWNAELGRKRAETDRVYLAAKQAINHLFVDYQDQQLNPEIGLAEINEASNLVKSISGVYSDTLLQIPGINYEIYTELSDRLQQASYLYTSRNAVQNGDFNSGLDSWNATTDASVQQDGSTHFLVLSHWDAQVSQQMRVNLNCKYVLRVTAKKVGGGDGYVTIRDGAHHQETLTFNACDYDVNGTYVNDNSYITKEVVFYPETKHMWVEVSESEGSFYIDSIEFIETQE

SEQ ID NO: 15 - protein, 1173 aa, Bacillus thuringiensis
MNRNNQGEYEIIDASTCGCSSDDVVQYPLARDPNAAFQNMNYKDYLKMSDGDYVDSYINPGLSIGRRDVTLTGVGIVALIVGTLGGPVGGIVTGLISSLLGLLWPSNDNDVWEAFMAQIEELIEQRIADQVVRNALDNLTGLRDYYNQYLLALEEWQERPNAVRSTLVFNRFETLHSHFVTSMPSFGSGPGSERYAVQLLTVYAQAANLHLLLLRDADIYGARWGLRESQIDLYFNELQNRTRDYTNHCVTAYNNGLEEIRGTSPASWLRYHQFRRETTLIALDLVAIFPYYNVREYPIGVNPQLTRDVYTDPIGVTFRREDWETGVECRPWVNTPYMSFSDLENAIIRPPHLFETLRNLTIHTGRYNLVGGARFIEGWVGHSVTNTRLGNSTVFTSNYGSLPPRFQVFNFTNFDVYQINTRADSTGTFRIPGFAVTRAQFIPGGTYSVAHRDPGACQQDYDSIEELPSLDPDEPINRSYSHRLSHVTLYKYTLSDTDYGVINYTDYGSMPAYVWTHRDVDLTNTITADRITQLPLVKASTLPAGTTVVKGPGFTGGDILRRTTNGTFGTLHVRVNSPLTQQYRLRVRFASTGNFSIRVLRGGTSIGDARFGSTMNRGQELTYESFVTREFTTTGPFNPPFTFTQTQEILTVNAEGVSTGGEYYIDSIEIVPVNPTREAEEDLEAAKKAVASLFTRTRDGLQVNVTDYQVDRAANLVLCLSDEQYAHDKKMLLEAVRAAKRLSRERNLLQDPDFNEINSTEDSGWKTSNGIIISEGGPFFKGRALQLASARENYPTYIYQKVDSSMLKPYTRYKLDGFVQSSQDLEIELIHHHKVHLVKNVPDNLVLDTYPDGSCNGINRCEEQQMVNSQLETEHHPMDCCEASQTHEFSSYIHTGDLNASVDQGIWVVLKIRTTDGSATLGNLELVEVGPLSGESLEREQRDNAKWNAELGRKRAEADRVYQGAKQAINHLFVDYQDQQLNPEVGLAEISEARNLIESISDVYCDAVLRIPGINYEMYTELSNRLQQAAYLYTSRNAVQNGDFNSGLDSWNATTDATVQQDGNMYFLVLSHWDAQVSQQFRVQPNCKYVLRVTAKKVGNGDGYVTIQDGAHHRETLTFNACDYDVNGTHVNDNSYITKELEFYPKTEHMWVEVSETEGTFYIDSIELIETQE

SEQ ID NO: 16 - protein, 1179 aa, Bacillus thuringiensis
MGGKSMNRNNQGEYEIIDASTCGCSSDDVVQYPLARDPNAAFQNMNYKDYLKMSDGDYVDSYINPGLSIGRRDVTLTGVGIVALIVGTLGGPVGGIVTGLISSLLGLLWPSNDNDVWEAFMAQIEELIEQRIADQVVRNALDNLTGLRDYYNQYLLALEEWQERPNAVRSTLVFNRFETLHSHFVTSMPSFGSGPGSERYAVQLLTVYAQAANLHLLLLRDADIYGARWGLRESQIDLYFNELQNRTRDYTNHCVTAYNNGLEEIRGTSPASWLRYHQFRRETTLIALDLVAIFPYYNVREYPIGVNPQLTRDVYTDPIGVTFRREDWETGVECRPWVNTPYMSFSDLENAIIRPPHLFETLRNLTIHTGRYNLVGGARFIEGWVGHSVTNTRLGNSTVFTSNYGSLPPRFQVFNFTNFDVYQINTRADSTGTFRIPGFAVTRAQFIPGGTYSVAHRDPGACQQDYDSIEELPSLDPDEPINRSYSHRLSHVTLYKYTLSDTDYGVINYTDYGSMPAYVWTHRDVDLTNTITADRITQLPLVKASTLPAGTTVVKGPGFTGGDILRRTTNGTFGTLHVRVNSPLTQQYRLRVRFASTGNFSIRVLRGGTSIGDARFGSTMNRGQELTYESFVTREFTTTGPFNPPFTFTQTQEILTVNAEGVSTGGEYYIDSIEIVPVNPTREAEEDLEAAKKAVASLFTRTRDGLQVNVTDYQVDQAANLVSCLSDEQYGYDKKMLLEAVRAAKRLSRERNLLQDPDFNTINSTEENGWKASNGVTISEGGPFYKGRALQLASARENYPTYIYQKVDASELKPYTRYRLDGFVKSSQDLEIDLIHHHKVHLVKNVPDNLVSDTYPDDSCSGINRCQEQQMVNAQLETEHHHPMDCCEAAQTHEFSSYIDTGDLNSSVDQGIWAIFKVRTTDGYATLGNLELVEVGPLSGESLEREQRDNTKWSAELGRKRAETDRVYQDAKQSINHLFVDYQDQQLNPEIGMADIMDAQNLVASISDVYSDAVLQIPGINYEIYTELSNRLQQASYLYTSRNAVQNGDFNNGLDSWNATAGASVQQDGNTHFLVLSHWDAQVSQQFRVQPNCKYVLRVTAEKVGGGDGYVTIRDGAHHTETLTFNACDYDINGTYVTDNTYLTKEVIFYSHTEHMWVEVNETEGAFHIDSIEFVETEK

SEQ ID NO: 17 - protein, 1147 aa, Artificial Sequence
  Mutant BT-0044
MDLDGNKTETETEIVNGSESSIDPSSVSYAGNNSYSSALNLNSCQNRGIAQWVNTLGGAIGQAVSIGTSIISLLAAPTLTGSISLAFNLIRRMGTGSNGSSISDLSICDLLSIINLRVSQAVLNDGIADFNGSVAVYDLYLHALRSWNNNPNAATAEELRTRFRIADSEFERILTRGSLTHGGSLARQDAQVLLLPSFVNAAYLHLLILRDASRYGASWGLFNTTPHINYPVRLQQLIGSYTHYCTHWYNQGLNEIRQRGNTAVNWLEFHRYRRDMTLMVLDVVSLFSALDTIRYPNATVVQLSRTVYTDPIGFVNRGSGNRLSWFDWRNQANFSTLESEMPTPSSPLSLNHMSIFTGPLTLPVSPNTHRARVWYGNQNMFTTGSQNSGQTTNSIQNISGLEIFRIDSQACNLNNNSYGVNRAEFFHGASQGSQRSVYQGYIRQSGLDNPVVMNLQSFLPGENSATPTAQDYTHILSNPVNIRGGLRQIVADRRSSVVVYGWTHKSLSRRSLVAPDQITQVPAVKASPSSHCTIIAGPGFTGGDLVSLQPNGQLVIPFQVSAPETNYHIRICYVSTSDCSINTICNDETHLSTLPSTTSSLENLQCNHLHYFNVGTFKPTIDSKLTLVNTSPNANIIIDKIEFIPVDTAQQQNEDLEAAKKAVASLFTRTRDGLQVNVKDYQVDQAANLVSCLSDEQYGYDKKMLLEAVRAAKRLSRERNLLQDPDFNTINSTEENGWKASNGVTISEGGPFYKGRAIQLASARENYPTYIYQKVDASELKPYTRYRLDGFVKSSQDLEIDLIHHHKVHLVKNVPDNLVSDTYPDDSCSGINRCQEQQMVNAQLETEHHHPMDCCEAAQTHEFSSYIDTGDLNSSVDQGIWAIFKVRTTDGYATLGNLELVEVGPLSGESLEREQRDNTKWSAELGRKRAETDRVYQDAKQSINHLFVDYQDQQLNPEIGMADIMDAQNLVASISDVYSDAVLQIPGINYEIYTELSNRLQQASYLYTSRNAVQNGDFNNGLDSWNATAGASVQQDGNTHFLVLSHWDAQVSQQFRVQPNCKYVLRVTAEKVGGGDGYVTIRDDAHHTETLTFNACDYDINGTYVTDNTYITKEVVFHPETQHMWVEVNETEGAFHLDSIEFVETEK

SEQ ID NO: 18 - protein, 1157 aa, Artificial Sequence
  Mutant BT-0051
MNRNNQNEYEIIDAPHCGCPSDDDVKYPLASDPNAALQNMNYKDYLQMTDEDYTDSYINPSLSISGRDAVQTALTVVGRILGALGVPFSGQIVSFYQFLLNTLWPVNDTAIWEAFMRQVEELVNQQITEFARNQALARLQGLGDSFNVYQRSLQNWLADRNDTRNLSVVRAQFIALDLDFVNAIPLFAVNGQQVPLLSVYAQAVNLHLLLLKDASLFGEGWGFTQGEISTHYDRQLELTARYTNYCETWYNTGLDRLRGTNTESWLRYHQFRREMTLVVLDVVALFPYYDVRLYPTGSNPQLTREVYTDPIVFNPPANVGLCRRWGTNPYNTFSELENAFIRPPHLFDRIQSLSISSNRFPVSSNFMDYWSGHTLRRSYLNDSAVQEDSYGLITTTRATINPGVDGTNRIESTAVDFRSALIGIYGVNRASFVPGGLFNGTTSPANGGCRDLYDTNDELPPDESTGSSTHRLSHVTFFSFQTNQAGSIANAGSVPTYVWTRRDVDLNNTITPNRITQLPLVKASAPVSGTTVLKGPGFTGGGILRRTTNGTFGTLRVTVNSPLTQQYRLRVRFASTGNFSIRLLRGGVSIGDVRLGSTMNRGQELTYESFFTREFTTTGPFNPPFTFTQAQEILTVNAEGVSTGGEYYIDRIEIVPVNPAREAEEDLEAAKKAVASLFTRTRDGLQVNVTDYQVDRAANLVSCLSDEQYSHDKKMLLEAVRAAKRLSRERNLLQDPDFNTINSTEENGWKASNGVTISEGGPFFKGRALQLASARENYPTYIYQKVDASVLKPYTRYRLDGFVKSSQDLEIDLIHHHKVHLVKNVPDNLVSDTYSDGSCSGINRCDEQQQVDMQLDAEHHPMDCCEAAQTHEFSSYINTGDLNASVDQGIWVVLKVRTTDGYATLGNLELVEVGPLSGESLEREQRDNAKWNAELGRKRAETDRVYLAAKQAINHLFVDYQDQQLNPEIGLAEINEASNLVKSISGVYSDTLLQIPGINYEIYTELSDRLQQASYLYTSRNAVQNGDFNSGLDSWNATTDASVQQDGSTHFLVLSHWDAQVSQQMRVNLNCKYVLRVTAKKVGGGDGYVTIRDGAHHQETLTFNACDYDVNGTYVNDNSYITKEVVFYPETKHMWVEVSESEGSFYIDSIEFIETQE

SEQ ID NO: 19 - protein, 1173 aa, Artificial Sequence; identical to SEQ ID NO: 15
  Mutant BT-0068

SEQ ID NO: 20 - protein, 1179 aa, Artificial Sequence
  Mutant BT-0128
MGGKSMNRNNQGEYEIIDASTCGCSSDDVVQYPLARDPNAAFQNMNYKDYLKMSDGDYVDSYINPGLSIGRRDVTLTGVGIVALIVGTLGGPVGGIVTGLISSLLGLLWPSNDNDVWEAFMAQIEELIEQRIADQVVRNALDNLTGLRDYYNQYLLALEEWQERPNAVRSTLVFNRFETLHSHFVTSMPSFGSGPGSERYAVQLLTVYAQAANLHLLLLRDADIYGARWGLRESQIDLYFNELQNRTRDYTNHCVTAYNNGLEEIRGTSPASWLRYHQFRRETTLIALDLVAIFPYYNVREYPIGVNPQLTRDVYTDPIGVTFRREDWETGVECRPWVNTPYMSFSDLENAIIRPPHLFETLRNLTIHTGRYNLVGGARFIEGWVGHSVTNTRLGNSTVFTSNYGSLPPRFQVFNFTNFDVYQINTRADSTGTFRIPGFAVTRAQFIPGGTYSVAHRDPGACQQDYDSIEELPSLDPDEPINRSYSHRLSHVTLYKYTLSDTDYGVINYTDYGSMPAYVWTHRDVDLTNTITADRITQLPLVKASTLPAGTTVVKGPGFTGGDILRRTTNGTFGTLHVRVNSPLTQQYRLRVRFASTGNFSIRVLRGGTSIGDARFGSTMNRGQELTYESFVTREFTTTGPFNPPFTFTQTQEILTVNAEGVSTGGEYYIDSIEIVPVNPTREAEEDLEAAKKAVASLFTRTRDGLQVNVTDYQVDQAANLVSCLSDEQYGYDKKMLLEAVRAAKRLSRERNLLQDPDFNTINSTEENGWKASNGVTISEGGPFYKGRALQLASARENYPTYIYQKVDASELKPYTRYRLDGFVKSSQDLEIDLIHHHKVHLVKNVPDNLVSDTYPDDSCSGINRCQEQQMVNAQLETEHHHPMDCCEAAQTHEFSSYIDTGDLNSSVDQGIWAIFKVRTTDGYATLGNLELVEVGPLSGESLEREQRDNTKWSAELGRKRAETDRVYQDAKQSINHLFVDYQDQQLNPEIGMADIMDAQNLVASISDVYSDAVLQIPGINYEIYTELSNRLQQASYLYTSRNAVQNGDFNNGLDSWNATAGASVQQDGNTHFLVLSHWDAQVSQQFRVQPNCKYVLRVTAEKVGGGDGYVTIRDGAHHTETLTFNACDYDINGTYVTDNTYLTKEVIFYSHTEHMWVEVNETEGAFHLDSLEFVETEK

SEQ ID NO: 21 - DNA, 26 bp, Artificial Sequence
  OAR2613a Forward Primer
aaacatgaaccgaaataatcaaaatg

SEQ ID NO: 22 - DNA, 22 bp, Artificial Sequence
  OAR2615a Reverse Primer
atccgtcccttgtgcgtgtaaa

SEQ ID NO: 23 - DNA, 30 bp, Artificial Sequence
  OAR2611a-F forward primer
gtttaaacatgaatcgaaataatcaaaatg

SEQ ID NO: 24 - DNA, 29 bp, Artificial Sequence
  OAR2612a-R reverse primer
ggcgcgccctactcttgtgtttcaataaa

SEQ ID NO: 25 - DNA, 29 bp, Artificial Sequence
  OAR2768-F forward primer
gtttaaacatgaatcaaaataaacacgga

SEQ ID NO: 26 - DNA, 31 bp, Artificial Sequence
  OAR2769-R reverse primer
ggcgcgccttactgttgggtttccatgaact